European Patent Application EP 4 365 586 A1, published May 8, 2024. Title: Antibody Analysis Method. Applicant: Shimadzu Corporation. The sequence listing filed with the application follows.

SEQUENCE LISTING (47 sequences)

SEQ ID NO: 1 - protein, 9 aa, Artificial Sequence
  Trastuzumab Signature peptides
IYPTNGYTR

SEQ ID NO: 2 - protein, 26 aa, Artificial Sequence
  Trastuzumab H-CDR3
WGGDGFYAMDYWGQGTLVTVSSASTK

SEQ ID NO: 3 - protein, 9 aa, Artificial Sequence
  Bevacizumab Signature peptides
FTFSLDTSK

SEQ ID NO: 4 - protein, 29 aa, Artificial Sequence
  Bevacizumab H-CDR3
YPHYYGSSHWYFDVWGQGTLVTVSSASTK

SEQ ID NO: 5 - protein, 6 aa, Artificial Sequence
  Cetuximab Signature peptides
SQVFFK

SEQ ID NO: 6 - protein, 26 aa, Artificial Sequence
  Cetuximab H-CDR3
ALTYYDYEFAYWGQGTLVTVSAASTK

SEQ ID NO: 7 - protein, 15 aa, Artificial Sequence
  Rituximab Signature peptides
ASGYTFTSYNMHWVK

SEQ ID NO: 8 - protein, 27 aa, Artificial Sequence
  Rituximab H-CDR3
STYYGGDWYFNVWGAGTTVTVSAASTK

SEQ ID NO: 9 - protein, 15 aa, Artificial Sequence
  Nivolumab Signature peptides
ASGITFSNSGMHWVR

SEQ ID NO: 10 - protein, 29 aa, Artificial Sequence
  Nivolumab H-CDR3
AEDTAVYYCATNDDWGQGTLVTVSSASTK

SEQ ID NO: 11 - protein, 16 aa, Artificial Sequence
  Brentuximab vedotin Signature peptides
VLIYAASNLESGIPAR

SEQ ID NO: 12 - protein, 54 aa, Artificial Sequence
  Brentuximab vedotin H-CDR3
ATLTVDTSSSTAFMQLSSLTSEDTAVYFCANYGNYWFAYWGQGTQVTVSAASTK

SEQ ID NO: 13 - protein, 16 aa, Artificial Sequence
  Pembrolizumab Signature peptides
LLIYLASYLESGVPAR

SEQ ID NO: 14 - protein, 22 aa, Artificial Sequence
  Pembrolizumab H-CDR3
FDMGFDYWGQGTTVTVSSASTK

SEQ ID NO: 15 - protein, 24 aa, Artificial Sequence
  Ipilimumab Signature peptides
TGWLGPFDYWGQGTLVTVSSASTK

SEQ ID NO: 16 - protein, 24 aa, Artificial Sequence
  Ipilimumab H-CDR3
TGWLGPFDYWGQGTLVTVSSASTK

SEQ ID NO: 17 - protein, 22 aa, Artificial Sequence
  Mogamulizumab Signature peptides
GLEWVATISSASTYSYYPDSVK

SEQ ID NO: 18 - protein, 25 aa, Artificial Sequence
  Mogamulizumab H-CDR3
HSDGNFAFGYWGQGTLVTVSSASTK

SEQ ID NO: 19 - protein, 11 aa, Artificial Sequence
  Ramucirumab Signature peptides
AFPPTFGGGTK

SEQ ID NO: 20 - protein, 22 aa, Artificial Sequence
  Ramucirumab H-CDR3
VTDAFDIWGQGTMVTVSSASTK

SEQ ID NO: 21 - protein, 22 aa, Artificial Sequence
  Atezolizumab Signature peptides
GLEWVAWISPYGGSTYYADSVK

SEQ ID NO: 22 - protein, 23 aa, Artificial Sequence
  Atezolizumab H-CDR3
HWPGGFDYWGQGTLVTVSSASTK

SEQ ID NO: 23 - protein, 18 aa, Artificial Sequence
  Durvalumab Signature peptides
VSSSYLAWYQQKPGQAPR

SEQ ID NO: 24 - protein, 27 aa, Artificial Sequence
  Durvalumab H-CDR3
EGGWFGELAFDYWGQGTLVTVSSASTK

SEQ ID NO: 25 - protein, 24 aa, Artificial Sequence
  Avelumab Signature peptides
LGTVTTVDYWGQGTLVTVSSASTK

SEQ ID NO: 26 - protein, 24 aa, Artificial Sequence
  Avelumab H-CDR3
LGTVTTVDYWGQGTLVTVSSASTK

SEQ ID NO: 27 - protein, 13 aa, Artificial Sequence
  Infliximab Signature peptides
SINSATHYAESVK

SEQ ID NO: 28 - protein, 24 aa, Artificial Sequence
  Infliximab H-CDR3
NYYGSTYDYWGQGTTLTVSSASTK

SEQ ID NO: 29 - protein, 5 aa, Artificial Sequence
  Tocilizumab Signature peptides
VTMLR

SEQ ID NO: 30 - protein, 21 aa, Artificial Sequence
  Tocilizumab H-CDR3
TTAMDYWGQGSLVTVSSASTK

SEQ ID NO: 31 - protein, 10 aa, Artificial Sequence
  Adalimumab Signature peptides
APYTFGQGTK

SEQ ID NO: 32 - protein, 27 aa, Artificial Sequence
  Adalimumab H-CDR3
VSYLSTASSLDYWGQGTLVTVSSASTK

SEQ ID NO: 33 - protein, 13 aa, Artificial Sequence
  Golimumab Signature peptides
SNWPPFTFGPGTK

SEQ ID NO: 34 - protein, 32 aa, Artificial Sequence
  Golimumab H-CDR3
DRGIAAGGNYYYYGMDVWGQGTTVTVSSASTK

SEQ ID NO: 35 - protein, 8 aa, Artificial Sequence
  Mepolizumab Signature peptides
DPPSSLLR

SEQ ID NO: 36 - protein, 8 aa, Artificial Sequence
  Mepolizumab H-CDR3
DPPSSLLR

SEQ ID NO: 37 - protein, 6 aa, Artificial Sequence
  Mepolizumab H-CDR3
LDYWGR

SEQ ID NO: 38 - protein, 12 aa, Artificial Sequence
  Mepolizumab H-CDR3
GTPVTVSSASTK

SEQ ID NO: 39 - protein, 12 aa, Artificial Sequence
  Mepolizumab H-CDR3
GPSVFPLAPSSK

SEQ ID NO: 40 - protein, 25 aa, Artificial Sequence
  Ustekinumab Signature peptides
RRPGQGYFDFWGQGTLVTVSSSSTK

SEQ ID NO: 41 - protein, 25 aa, Artificial Sequence
  Ustekinumab H-CDR3
RRPGQGYFDFWGQGTLVTVSSSSTK

SEQ ID NO: 42 - protein, 16 aa, Artificial Sequence
  Eculizumab Signature peptides
LLIYGATNLADGVPSR

SEQ ID NO: 43 - protein, 28 aa, Artificial Sequence
  Eculizumab H-CDR3
YFFGSSPNWYFDVWGQGTLVTVSSASTK

SEQ ID NO: 44 - protein, 14 aa, Artificial Sequence
  Abatacept Signature peptides
MHVAQPAVVLASSR

SEQ ID NO: 45 - protein, 6 aa, Artificial Sequence
  Aflibercept Signature peptides
IIWDSR

SEQ ID NO: 46 - protein, 5 aa, Artificial Sequence
  Etanercept Signature peptides
VFCTK

SEQ ID NO: 47 - protein, 15 aa, Artificial Sequence
  P14R
PPPPPPPPPPPPPPR